European Patent Specification EP 3 651 566 B1, published June 5, 2024. Title: POWDERY MILDEW RESISTANT ROSE. Applicant: Dümmen Group BV. The sequence listing filed with the application follows.

SEQUENCE LISTING (2 sequences)

SEQ ID NO: 1 - DNA, 52 bp, Rosa
tttgttcattataaactcattcctcgcttcctcaaccttctctgaaacgacc

SEQ ID NO: 2 - DNA, 50 bp, Rosa
ggcttttcgccctgcgtcttgctctccaaaaactcactactaatttgtca